European Patent Application EP 4 692 332 A1, published February 11, 2026. Title: Method for producing megakaryocytes. Applicant: 大塚製薬株式会社. The sequence listing filed with the application follows.

SEQUENCE LISTING (3 sequences)

SEQ ID NO: 1 - DNA, 947 bp, Homo sapiens
  source 1..947: mol_type = genomic DNA
gtgaacggaccaagagtaaacagtgtgctcaatgctgtgcctacgtgtgttagcccacgcggccagcctgaggagtcagggaaggctcccctaggcaaagcccccaaccagaatcaagtcttaatggttaaagagctccatcacccaaaaaggattgagggcctaccttcaactgaacagctaatgcataatctcagaaactgtgagtcaaaattccctggaataactccactttatccccaatctccttgccacctagaccaaggtccattcaccaccctgtccccagcactgactgcactgctgtggccacactaaagcttggctcaagacggaggaggagtgaggaagctgctgcaccaatatggctggttgaggccgcccaaggtcctagaaggaggaagtgggtaaatgccatatccaaaaagatacagaagcctcaggttttatcgggggcagcagcttccttctccttccccgacctgtggccaagtcacaaagcaccacagctgtacagccagatgggggaagggaggagattagaactgtaggctagagtagacaagtatggaccagttcacaatcacgctatcccaagcagaaagtgatggtggcttggactagcacggtggtagtagagatggggtaaagattcaagagacatcattgataggcagaaccaataggacatggtaataaactattctcaggaaaggggaggagtcatggctttcagccatgagcatccaccctctgggtggcctcacccacttcctggcaattctagccaccatgagtccaggggctatagccctttgctctgcccgttgctcagcaagttacttggggttccagtttgataagaaaagacttcctgtggaggaatctgaagggaaggaggaggagctggcccattcctgcctgggaggttgtggaagaaggaagat

SEQ ID NO: 2 - DNA, 1908 bp, Homo sapiens
  source 1..1908: mol_type = genomic DNA
atgccctcctgggccctcttcatggtcacctcctgcctcctcctggcccctcaaaacctggcccaagtcagcagccaagatgtctccttgctggcatcagactcagagcccctgaagtgtttctcccgaacatttgaggacctcacttgcttctgggatgaggaagaggcagcgcccagtgggacataccagctgctgtatgcctacccgcgggagaagccccgtgcttgccccctgagttcccagagcatgccccactttggaacccgatacgtgtgccagtttccagaccaggaggaagtgcgtctcttctttccgctgcacctctgggtgaagaatgtgttcctaaaccagactcggactcagcgagtcctctttgtggacagtgtaggcctgccggctccccccagtatcatcaaggccatgggtgggagccagccaggggaacttcagatcagctgggaggagccagctccagaaatcagtgatttcctgaggtacgaactccgctatggccccagagatcccaagaactccactggtcccacggtcatacagctgattgccacagaaacctgctgccctgctctgcagaggcctcactcagcctctgctctggaccagtctccatgtgctcagcccacaatgccctggcaagatggaccaaagcagacctccccaagtagagaagcttcagctctgacagcagagggtggaagctgcctcatctcaggactccagcctggcaactcctactggctgcagctgcgcagcgaacctgatgggatctccctcggtggctcctggggatcctggtccctccctgtgactgtggacctgcctggagatgcagtggcacttggactgcaatgctttaccttggacctgaagaatgttacctgtcaatggcagcaacaggaccatgctagctcccaaggcttcttctaccacagcagggcacggtgctgccccagagacaggtaccccatctgggagaactgcgaagaggaagagaaaacaaatccaggactacagaccccacagttctctcgctgccacttcaagtcacgaaatgacagcattattcacatccttgtggaggtgaccacagccccgggtactgttcacagctacctgggctcccctttctggatccaccaggctgtgcgcctccccaccccaaacttgcactggagggagatctccagtgggcatctggaattggagtggcagcacccatcgtcctgggcagcccaagagacctgttatcaactccgatacacaggagaaggccatcaggactggaaggtgctggagccgcctctcggggcccgaggagggaccctggagctgcgcccgcgatctcgctaccgtttacagctgcgcgccaggctcaacggccccacctaccaaggtccctggagctcgtggtcggacccaactagggtggagaccgccaccgagaccgcctggatctccttggtgaccgctctgcatctagtgctgggcctcagcgccgtcctgggcctgctgctgctgaggtggcagtttcctgcacactacaggagactgaggcatgccctgtggccctcacttccagacctgcaccgggtcctaggccagtaccttagggacactgcagccctgagcccgcccaaggccacagtctcagatacctgtgaagaagtggaacccagcctccttgaaatcctccccaagtcctcagagaggactcctttgcccctgtgttcctcccaggcccagatggactaccgaagattgcagccttcttgcctggggaccatgcccctgtctgtgtgcccacccatggctgagtcagggtcctgctgtaccacccacattgccaaccattcctacctaccactaagctattggcagcagccttga

SEQ ID NO: 3 - DNA, 2867 bp, synthetic construct
  source 1..2867: mol_type = other DNA
gtgaacggaccaagagtaaacagtgtgctcaatgctgtgcctacgtgtgttagcccacgcggccagcctgaggagtcagggaaggctcccctaggcaaagcccccaaccagaatcaagtcttaatggttaaagagctccatcacccaaaaaggattgagggcctaccttcaactgaacagctaatgcataatctcagaaactgtgagtcaaaattccctggaataactccactttatccccaatctccttgccacctagaccaaggtccattcaccaccctgtccccagcactgactgcactgctgtggccacactaaagcttggctcaagacggaggaggagtgaggaagctgctgcaccaatatggctggttgaggccgcccaaggtcctagaaggaggaagtgggtaaatgccatatccaaaaagatacagaagcctcaggttttatcgggggcagcagcttccttctccttccccgacctgtggccaagtcacaaagcaccacagctgtacagccagatgggggaagggaggagattagaactgtaggctagagtagacaagtatggaccagttcacaatcacgctatcccaagcagaaagtgatggtggcttggactagcacggtggtagtagagatggggtaaagattcaagagacatcattgataggcagaaccaataggacatggtaataaactattctcaggaaaggggaggagtcatggctttcagccatgagcatccaccctctgggtggcctcacccacttcctggcaattctagccaccatgagtccaggggctatagccctttgctctgcccgttgctcagcaagttacttggggttccagtttgataagaaaagacttcctgtggaggaatctgaagggaaggaggaggagctggcccattcctgcctgggaggttgtggaagaaggaagataccggtgccaccatgccctcctgggccctcttcatggtcacctcctgcctcctcctggcccctcaaaacctggcccaagtcagcagccaagatgtctccttgctggcatcagactcagagcccctgaagtgtttctcccgaacatttgaggacctcacttgcttctgggatgaggaagaggcagcgcccagtgggacataccagctgctgtatgcctacccgcgggagaagccccgtgcttgccccctgagttcccagagcatgccccactttggaacccgatacgtgtgccagtttccagaccaggaggaagtgcgtctcttctttccgctgcacctctgggtgaagaatgtgttcctaaaccagactcggactcagcgagtcctctttgtggacagtgtaggcctgccggctccccccagtatcatcaaggccatgggtgggagccagccaggggaacttcagatcagctgggaggagccagctccagaaatcagtgatttcctgaggtacgaactccgctatggccccagagatcccaagaactccactggtcccacggtcatacagctgattgccacagaaacctgctgccctgctctgcagaggcctcactcagcctctgctctggaccagtctccatgtgctcagcccacaatgccctggcaagatggaccaaagcagacctccccaagtagagaagcttcagctctgacagcagagggtggaagctgcctcatctcaggactccagcctggcaactcctactggctgcagctgcgcagcgaacctgatgggatctccctcggtggctcctggggatcctggtccctccctgtgactgtggacctgcctggagatgcagtggcacttggactgcaatgctttaccttggacctgaagaatgttacctgtcaatggcagcaacaggaccatgctagctcccaaggcttcttctaccacagcagggcacggtgctgccccagagacaggtaccccatctgggagaactgcgaagaggaagagaaaacaaatccaggactacagaccccacagttctctcgctgccacttcaagtcacgaaatgacagcattattcacatccttgtggaggtgaccacagccccgggtactgttcacagctacctgggctcccctttctggatccaccaggctgtgcgcctccccaccccaaacttgcactggagggagatctccagtgggcatctggaattggagtggcagcacccatcgtcctgggcagcccaagagacctgttatcaactccgatacacaggagaaggccatcaggactggaaggtgctggagccgcctctcggggcccgaggagggaccctggagctgcgcccgcgatctcgctaccgtttacagctgcgcgccaggctcaacggccccacctaccaaggtccctggagctcgtggtcggacccaactagggtggagaccgccaccgagaccgcctggatctccttggtgaccgctctgcatctagtgctgggcctcagcgccgtcctgggcctgctgctgctgaggtggcagtttcctgcacactacaggagactgaggcatgccctgtggccctcacttccagacctgcaccgggtcctaggccagtaccttagggacactgcagccctgagcccgcccaaggccacagtctcagatacctgtgaagaagtggaacccagcctccttgaaatcctccccaagtcctcagagaggactcctttgcccctgtgttcctcccaggcccagatggactaccgaagattgcagccttcttgcctggggaccatgcccctgtctgtgtgcccacccatggctgagtcagggtcctgctgtaccacccacattgccaaccattcctacctaccactaagctattggcagcagccttga